European Patent Application EP 4 231 017 A1, published August 23, 2023. Title: DETECTION AND QUANTIFICATION OF ANTI-DRUG ANTIBODIES AND ANTI-SELF ANTIBODIES. Applicant: PROMISE PROTEOMICS. The sequence listing filed with the application follows.

SEQUENCE LISTING (3 sequences)

SEQ ID NO: 1 - protein, 13 aa, Artificial Sequence
  Tryptic Proteotypic peptide from Infliximab
SINSATHYAESVK

SEQ ID NO: 2 - protein, 10 aa, Artificial Sequence
  Tryptic Proteotypic peptide from Adalimumab
APYTFGQGTK

SEQ ID NO: 3 - protein, 15 aa, Artificial Sequence
  Tryptic Proteotypic peptide from Infliximab
ASQFVGSSIHWYQQR